European Patent Application EP 4 206 325 A1, published July 5, 2023. Title: A novel nucleic acid molecule that supresses expression of a target gene. Applicant: BONAC CORPORATION. The sequence listing filed with the application follows.

SEQUENCE LISTING (533 sequences)

SEQ ID NO: 1 - RNA, 21 nt, Artificial Sequence
  Nucleic acid sequence used for crosslinking
gauaagaugaaucucuucucc

SEQ ID NO: 2 - RNA, 21 nt, Artificial Sequence
  Nucleic acid sequence used for crosslinking
agaagagauucaucuuaucuc

SEQ ID NO: 3 - RNA, 22 nt, Artificial Sequence
  Nucleic acid sequence used for crosslinking
agauaagaugaaucucuucucc

SEQ ID NO: 4 - RNA, 25 nt, Artificial Sequence
  Nucleic acid sequence used for crosslinking
uggagauaagaugaaucucuucucc

SEQ ID NO: 5 - RNA, 23 nt, Artificial Sequence
  Nucleic acid sequence used for crosslinking
agaagagauucaucuuaucucca

SEQ ID NO: 6 - RNA, 22 nt, Artificial Sequence
  Nucleic acid sequence used for crosslinking
aguaaagaugaaucucuucucc

SEQ ID NO: 7 - RNA, 20 nt, Artificial Sequence
  Nucleic acid sequence used for crosslinking
auaagaugaaucucuucucc

SEQ ID NO: 8 - RNA, 18 nt, Artificial Sequence
  Nucleic acid sequence used for crosslinking
agaagagauucaucuuau

SEQ ID NO: 9 - RNA, 22 nt, Artificial Sequence
  Nucleic acid sequence used for crosslinking
ugauaagaugaaucucuucucc

SEQ ID NO: 10 - RNA, 20 nt, Artificial Sequence
  nucleic acid sequence used for crosslinking
agaagagauucaucuuaucu

SEQ ID NO: 11 - RNA, 23 nt, Artificial Sequence
  Nucleic acid sequence used for crosslinking
uagauaagaugaaucucuucucc

SEQ ID NO: 12 - RNA, 21 nt, Artificial Sequence
  Nucleic acid sequence used for crosslinking
agaagagauucaucuuaucuu

SEQ ID NO: 13 - RNA, 21 nt, Artificial Sequence
  Nucleic acid sequence used for crosslinking
uauaagaugaaucucuucucc

SEQ ID NO: 14 - RNA, 21 nt, Artificial Sequence
  Nucleic acid sequence used for crosslinking
agaagagauucaucuuauauu

SEQ ID NO: 15 - RNA, 20 nt, Artificial Sequence
  Nucleic acid sequence used for crosslinking
agaagagauucaucuuauau

SEQ ID NO: 16 - RNA, 22 nt, Artificial Sequence
  Nucleic acid sequence used for crosslinking
agaagagauucaucuuaucucc

SEQ ID NO: 17 - RNA, 20 nt, Artificial Sequence
  Nucleic acid sequence used for crosslinking
uuuguuggauuugaaauucc

SEQ ID NO: 18 - RNA, 20 nt, Artificial Sequence
  Nucleic acid sequence used for crosslinking
aauuucaaauccaacaaagu

SEQ ID NO: 19 - RNA, 20 nt, Artificial Sequence
  Nucleic acid sequence used for crosslinking
uggucguauugggcgccugg

SEQ ID NO: 20 - RNA, 20 nt, Artificial Sequence
  Nucleic acid sequence used for crosslinking
aggcgcccaauacgaccaaa

SEQ ID NO: 21 - RNA, 20 nt, Artificial Sequence
  Nucleic acid sequence used for crosslinking
uggucguauugggcgccugg

SEQ ID NO: 22 - RNA, 20 nt, Artificial Sequence
  Nucleic acid sequence used for crosslinking
aggcgcccaauacgaccaaa

SEQ ID NO: 23 - RNA, 21 nt, Artificial Sequence
  Nucleic acid sequence used for crosslinking
uuggucguauugggcgccugg

SEQ ID NO: 24 - RNA, 21 nt, Artificial Sequence
  Nucleic acid sequence used for crosslinking
aggcgcccaauacgaccaaau

SEQ ID NO: 25 - RNA, 21 nt, Artificial Sequence
  Nucleic acid sequence used for crosslinking
uuggucguauugggcgccugg

SEQ ID NO: 26 - RNA, 21 nt, Artificial Sequence
  Nucleic acid sequence used for crosslinking
aggcgcccaauacgaccaaau

SEQ ID NO: 27 - RNA, 21 nt, Artificial Sequence
  Nucleic acid sequence used for crosslinking
  modified_base (3)..(3): um
  modified_base (11)..(11): um
  modified_base (13)..(13): um
  modified_base (18)..(18): um
cuuuguuggauuugaaauucc

SEQ ID NO: 28 - RNA, 21 nt, Artificial Sequence
  Nucleic acid sequence used for crosslinking
  modified_base (4)..(4): um
  modified_base (6)..(6): cm
  modified_base (10)..(10): um
  modified_base (12)..(12): cm
  modified_base (15)..(15): cm
aauuucaaauccaacaaaguc

SEQ ID NO: 29 - RNA, 21 nt, Artificial Sequence
  Nucleic acid sequence used for crosslinking
cuuuguuggauuugaaauucc

SEQ ID NO: 30 - RNA, 21 nt, Artificial Sequence
  Nucleic acid sequence used for crosslinking
aauuucaaauccaacaaaguc

SEQ ID NO: 31 - RNA, 21 nt, Artificial Sequence
  Nucleic acid sequence used for crosslinking
uuauggguugggacuaccuua

SEQ ID NO: 32 - RNA, 21 nt, Artificial Sequence
  Nucleic acid sequence used for crosslinking
ggguagucccaacccauaagg

SEQ ID NO: 33 - RNA, 22 nt, Artificial Sequence
  Nucleic acid sequence used for crosslinking
uuuggucguauugggcgccugg

SEQ ID NO: 34 - RNA, 22 nt, Artificial Sequence
  Nucleic acid sequence used for crosslinking
aggcgcccaauacgaccaaauc

SEQ ID NO: 35 - RNA, 22 nt, Artificial Sequence
  Nucleic acid sequence used for crosslinking
gauuuggucguauugggcgccu

SEQ ID NO: 36 - RNA, 22 nt, Artificial Sequence
  Nucleic acid sequence used for crosslinking
gcgcccaauacgaccaaauccg

SEQ ID NO: 37 - RNA, 22 nt, Artificial Sequence
  Nucleic acid sequence used for crosslinking
cgucaaggcugagaacgggaag

SEQ ID NO: 38 - RNA, 22 nt, Artificial Sequence
  Nucleic acid sequence used for crosslinking
ucccguucucagccuugacggu

SEQ ID NO: 39 - RNA, 22 nt, Artificial Sequence
  Nucleic acid sequence used for crosslinking
cacuccuccaccuuugacgcug

SEQ ID NO: 40 - RNA, 22 nt, Artificial Sequence
  Nucleic acid sequence used for crosslinking
gcgucaaagguggaggaguggg

SEQ ID NO: 41 - RNA, 22 nt, Artificial Sequence
  Nucleic acid sequence used for crosslinking
uuuggucguauugggcgccugg

SEQ ID NO: 42 - RNA, 22 nt, Artificial Sequence
  Nucleic acid sequence used for crosslinking
aggcgcccaauacgaccaaauc

SEQ ID NO: 43 - RNA, 22 nt, Artificial Sequence
  Nucleic acid sequence used for crosslinking
auggggaaggugaaggucggag

SEQ ID NO: 44 - RNA, 22 nt, Artificial Sequence
  Nucleic acid sequence used for crosslinking
ccgaccuucaccuuccccaugg

SEQ ID NO: 45 - RNA, 22 nt, Artificial Sequence
  Nucleic acid sequence used for crosslinking
ggugaagcaggcgucggagggc

SEQ ID NO: 46 - RNA, 22 nt, Artificial Sequence
  Nucleic acid sequence used for crosslinking
ccuccgacgccugcuucaccac

SEQ ID NO: 47 - RNA, 22 nt, Artificial Sequence
  Nucleic acid sequence used for crosslinking
cugacuucaacagcgacaccca

SEQ ID NO: 48 - RNA, 22 nt, Artificial Sequence
  Nucleic acid sequence used for crosslinking
ggugucgcuguugaagucagag

SEQ ID NO: 49 - RNA, 22 nt, Artificial Sequence
  Nucleic acid sequence used for crosslinking
uggugaagcaggcgucggaggg

SEQ ID NO: 50 - RNA, 22 nt, Artificial Sequence
  Nucleic acid sequence used for crosslinking
cuccgacgccugcuucaccacc

SEQ ID NO: 51 - RNA, 22 nt, Artificial Sequence
  Nucleic acid sequence used for crosslinking
uggggaaggugaaggucggagu

SEQ ID NO: 52 - RNA, 22 nt, Artificial Sequence
  Nucleic acid sequence used for crosslinking
uccgaccuucaccuuccccaug

SEQ ID NO: 53 - RNA, 22 nt, Artificial Sequence
  Nucleic acid sequence used for crosslinking
cuccuccaccuuugacgcuggg

SEQ ID NO: 54 - RNA, 22 nt, Artificial Sequence
  Nucleic acid sequence used for crosslinking
cagcgucaaagguggaggagug

SEQ ID NO: 55 - RNA, 22 nt, Artificial Sequence
  Nucleic acid sequence used for crosslinking
ccuccgggaaacuguggcguga

SEQ ID NO: 56 - RNA, 22 nt, Artificial Sequence
  Nucleic acid sequence used for crosslinking
acgccacaguuucccggagggg

SEQ ID NO: 57 - RNA, 22 nt, Artificial Sequence
  Nucleic acid sequence used for crosslinking
acuccuccaccuuugacgcugg

SEQ ID NO: 58 - RNA, 22 nt, Artificial Sequence
  Nucleic acid sequence used for crosslinking
agcgucaaagguggaggagugg

SEQ ID NO: 59 - RNA, 22 nt, Artificial Sequence
  Nucleic acid sequence used for crosslinking
ggcgcugaguacgucguggagu

SEQ ID NO: 60 - RNA, 22 nt, Artificial Sequence
  Nucleic acid sequence used for crosslinking
uccacgacguacucagcgccag

SEQ ID NO: 61 - RNA, 22 nt, Artificial Sequence
  Nucleic acid sequence used for crosslinking
aaaucaaguggggcgaugcugg

SEQ ID NO: 62 - RNA, 22 nt, Artificial Sequence
  Nucleic acid sequence used for crosslinking
agcaucgccccacuugauuuug

SEQ ID NO: 63 - RNA, 22 nt, Artificial Sequence
  Nucleic acid sequence used for crosslinking
cugaugcccccauguucgucau

SEQ ID NO: 64 - RNA, 22 nt, Artificial Sequence
  Nucleic acid sequence used for crosslinking
gacgaacaugggggcaucagca

SEQ ID NO: 65 - RNA, 22 nt, Artificial Sequence
  Nucleic acid sequence used for crosslinking
ggaaggugaaggucggagucaa

SEQ ID NO: 66 - RNA, 22 nt, Artificial Sequence
  Nucleic acid sequence used for crosslinking
gacuccgaccuucaccuucccc

SEQ ID NO: 67 - RNA, 22 nt, Artificial Sequence
  Nucleic acid sequence used for crosslinking
gcugaugcccccauguucguca

SEQ ID NO: 68 - RNA, 22 nt, Artificial Sequence
  Nucleic acid sequence used for crosslinking
acgaacaugggggcaucagcag

SEQ ID NO: 69 - RNA, 22 nt, Artificial Sequence
  Nucleic acid sequence used for crosslinking
ugaugcccccauguucgucaug

SEQ ID NO: 70 - RNA, 22 nt, Artificial Sequence
  Nucleic acid sequence used for crosslinking
ugacgaacaugggggcaucagc

SEQ ID NO: 71 - RNA, 22 nt, Artificial Sequence
  Nucleic acid sequence used for crosslinking
caaaaucaaguggggcgaugcu

SEQ ID NO: 72 - RNA, 22 nt, Artificial Sequence
  Nucleic acid sequence used for crosslinking
caucgccccacuugauuuugga

SEQ ID NO: 73 - RNA, 22 nt, Artificial Sequence
  Nucleic acid sequence used for crosslinking
ccaaggucauccaugacaacuu

SEQ ID NO: 74 - RNA, 22 nt, Artificial Sequence
  Nucleic acid sequence used for crosslinking
guugucauggaugaccuuggcc

SEQ ID NO: 75 - RNA, 22 nt, Artificial Sequence
  Nucleic acid sequence used for crosslinking
aaauuccauggcaccgucaagg

SEQ ID NO: 76 - RNA, 22 nt, Artificial Sequence
  Nucleic acid sequence used for crosslinking
uugacggugccauggaauuugc

SEQ ID NO: 77 - RNA, 22 nt, Artificial Sequence
  Nucleic acid sequence used for crosslinking
caacggauuuggucguauuggg

SEQ ID NO: 78 - RNA, 22 nt, Artificial Sequence
  Nucleic acid sequence used for crosslinking
caauacgaccaaauccguugac

SEQ ID NO: 79 - RNA, 22 nt, Artificial Sequence
  Nucleic acid sequence used for crosslinking
ccugguaugacaacgaauuugg

SEQ ID NO: 80 - RNA, 22 nt, Artificial Sequence
  Nucleic acid sequence used for crosslinking
aaauucguugucauaccaggaa

SEQ ID NO: 81 - RNA, 22 nt, Artificial Sequence
  Nucleic acid sequence used for crosslinking
  modified_base (21)..(21): 2'-F modified
  misc_feature (22)..(22): DNA
uuuggucguauugggcgccugg

SEQ ID NO: 82 - RNA, 22 nt, Artificial Sequence
  Nucleic acid sequence used for crosslinking
aggcgcccaauacgaccaaauc

SEQ ID NO: 83 - RNA, 22 nt, Artificial Sequence
  Nucleic acid sequence used for crosslinking
acuuuguuggauuugaaauucc

SEQ ID NO: 84 - RNA, 22 nt, Artificial Sequence
  Nucleic acid sequence used for crosslinking
aauuucaaauccaacaaagucu

SEQ ID NO: 85 - RNA, 22 nt, Artificial Sequence
  Nucleic acid sequence used for crosslinking
cuuauggguugggacuaccuua

SEQ ID NO: 86 - RNA, 22 nt, Artificial Sequence
  Nucleic acid sequence used for crosslinking
ggguagucccaacccauaaggu

SEQ ID NO: 87 - RNA, 18 nt, Artificial Sequence
  Nucleic acid sequence used for crosslinking
aagaugaaucucuucucc

SEQ ID NO: 88 - RNA, 18 nt, Artificial Sequence
  Nucleic acid sequence used for crosslinking
agaagagauucaucuuau

SEQ ID NO: 89 - RNA, 18 nt, Artificial Sequence
  Nucleic acid sequence used for crosslinking
aagaugaaucucuucucc

SEQ ID NO: 90 - RNA, 18 nt, Artificial Sequence
  Nucleic acid sequence used for crosslinking
agaagagauucaucuuau

SEQ ID NO: 91 - RNA, 18 nt, Artificial Sequence
  Nucleic acid sequence used for crosslinking
aagaugaaucucuucucc

SEQ ID NO: 92 - RNA, 18 nt, Artificial Sequence
  Nucleic acid sequence used for crosslinking
agaagagauucaucuuau

SEQ ID NO: 93 - RNA, 19 nt, Artificial Sequence
  Nucleic acid sequence used for crosslinking
uaagaugaaucucuucucc

SEQ ID NO: 94 - RNA, 19 nt, Artificial Sequence
  Nucleic acid sequence used for crosslinking
agaagagauucaucuuauc

SEQ ID NO: 95 - RNA, 19 nt, Artificial Sequence
  Nucleic acid sequence used for crosslinking
ggucguauugggcgccugg

SEQ ID NO: 96 - RNA, 19 nt, Artificial Sequence
  Nucleic acid sequence used for crosslinking
aggcgcccaauacgaccaa

SEQ ID NO: 97 - RNA, 19 nt, Artificial Sequence
  Nucleic acid sequence used for crosslinking
uaagaugaaucucuucucc

SEQ ID NO: 98 - RNA, 19 nt, Artificial Sequence
  Nucleic acid sequence used for crosslinking
agaagagauucaucuuauc

SEQ ID NO: 99 - RNA, 19 nt, Artificial Sequence
  Nucleic acid sequence used for crosslinking
uaagaugaaucucuucucc

SEQ ID NO: 100 - RNA, 19 nt, Artificial Sequence
  Nucleic acid sequence used for crosslinking
agaagagauucaucuuauc

SEQ ID NO: 101 - RNA, 19 nt, Artificial Sequence
  Nucleic acid sequence used for crosslinking
uuguuggauuugaaauucc

SEQ ID NO: 102 - RNA, 19 nt, Artificial Sequence
  Nucleic acid sequence used for crosslinking
aauuucaaauccaacaaag

SEQ ID NO: 103 - RNA, 23 nt, Artificial Sequence
  Nucleic acid sequence used for crosslinking
gagauaagaugaaucucuucucc

SEQ ID NO: 104 - RNA, 23 nt, Artificial Sequence
  Nucleic acid sequence used for crosslinking
agaagagauucaucuuaucucca

SEQ ID NO: 105 - RNA, 23 nt, Artificial Sequence
  Nucleic acid sequence used for crosslinking
auuuggucguauugggcgccugg

SEQ ID NO: 106 - RNA, 23 nt, Artificial Sequence
  Nucleic acid sequence used for crosslinking
aggcgcccaauacgaccaaaucc

SEQ ID NO: 107 - RNA, 23 nt, Artificial Sequence
  Nucleic acid sequence used for crosslinking
gagauaagaugaaucucuucucc

SEQ ID NO: 108 - RNA, 23 nt, Artificial Sequence
  Nucleic acid sequence used for crosslinking
agaagagauucaucuuaucucca

SEQ ID NO: 109 - RNA, 23 nt, Artificial Sequence
  Nucleic acid sequence used for crosslinking
auuuggucguauugggcgccugg

SEQ ID NO: 110 - RNA, 23 nt, Artificial Sequence
  Nucleic acid sequence used for crosslinking
aggcgcccaauacgaccaaaucc

SEQ ID NO: 111 - RNA, 23 nt, Artificial Sequence
  Nucleic acid sequence used for crosslinking
gagauaagaugaaucucuucucc

SEQ ID NO: 112 - RNA, 23 nt, Artificial Sequence
  Nucleic acid sequence used for crosslinking
agaagagauucaucuuaucucca

SEQ ID NO: 113 - RNA, 23 nt, Artificial Sequence
  Nucleic acid sequence used for crosslinking
auuuggucguauugggcgccugg

SEQ ID NO: 114 - RNA, 23 nt, Artificial Sequence
  Nucleic acid sequence used for crosslinking
aggcgcccaauacgaccaaaucc

SEQ ID NO: 115 - RNA, 24 nt, Artificial Sequence
  Nucleic acid sequence used for crosslinking
ggagauaagaugaaucucuucucc

SEQ ID NO: 116 - RNA, 24 nt, Artificial Sequence
  Nucleic acid sequence used for crosslinking
agaagagauucaucuuaucuccau

SEQ ID NO: 117 - RNA, 24 nt, Artificial Sequence
  Nucleic acid sequence used for crosslinking
ggagauaagaugaaucucuucucc

SEQ ID NO: 118 - RNA, 24 nt, Artificial Sequence
  Nucleic acid sequence used for crosslinking
agaagagauucaucuuaucuccau

SEQ ID NO: 119 - RNA, 24 nt, Artificial Sequence
  Nucleic acid sequence used for crosslinking
ggagauaagaugaaucucuucucc

SEQ ID NO: 120 - RNA, 24 nt, Artificial Sequence
  Nucleic acid sequence used for crosslinking
agaagagauucaucuuaucuccau

SEQ ID NO: 121 - RNA, 24 nt, Artificial Sequence
  Nucleic acid sequence used for crosslinking
agacuuuguuggauuugaaauucc

SEQ ID NO: 122 - RNA, 24 nt, Artificial Sequence
  Nucleic acid sequence used for crosslinking
aauuucaaauccaacaaagucugg

SEQ ID NO: 123 - RNA, 21 nt, Artificial Sequence
  Nucleic acid sequence used for crosslinking
gauaagaugaaucucuucucc

SEQ ID NO: 124 - RNA, 21 nt, Artificial Sequence
  Nucleic acid sequence used for crosslinking
agaagagauucaucuuaucuc

SEQ ID NO: 125 - RNA, 22 nt, Artificial Sequence
  Nucleic acid sequence used for crosslinking
agauaagaugaaucucuucucc

SEQ ID NO: 126 - RNA, 22 nt, Artificial Sequence
  Nucleic acid sequence used for crosslinking
agaagagauucaucuuaucucc

SEQ ID NO: 127 - RNA, 22 nt, Artificial Sequence
  Nucleic acid sequence used for crosslinking
uuuggucguauugggcgccugg

SEQ ID NO: 128 - RNA, 22 nt, Artificial Sequence
  Nucleic acid sequence used for crosslinking
aggcgcccaauacgaccaaauc

SEQ ID NO: 129 - RNA, 22 nt, Artificial Sequence
  Nucleic acid sequence used for crosslinking
agauaagaugaaucucuucucc

SEQ ID NO: 130 - RNA, 22 nt, Artificial Sequence
  Nucleic acid sequence used for crosslinking
agaagagauucaucuuaucucc

SEQ ID NO: 131 - RNA, 21 nt, Artificial Sequence
  Nucleic acid sequence used for crosslinking
gauaagaugaaucucuucucc

SEQ ID NO: 132 - RNA, 21 nt, Artificial Sequence
  Nucleic acid sequence used for crosslinking
agaagagauucaucuuaucuc

SEQ ID NO: 133 - RNA, 22 nt, Artificial Sequence
  Nucleic acid sequence used for crosslinking
acuuuguuggauuugaaauucc

SEQ ID NO: 134 - RNA, 22 nt, Artificial Sequence
  Nucleic acid sequence used for crosslinking
aauuucaaauccaacaaagucu

SEQ ID NO: 135 - RNA, 21 nt, Artificial Sequence
  Nucleic acid sequence used for crosslinking
gauaagaugaaucucuucucc

SEQ ID NO: 136 - RNA, 21 nt, Artificial Sequence
  Nucleic acid sequence used for crosslinking
agaagagauucaucuuaucuc

SEQ ID NO: 137 - RNA, 22 nt, Artificial Sequence
  Nucleic acid sequence used for crosslinking
uuuggucguauugggcgccugg

SEQ ID NO: 138 - RNA, 22 nt, Artificial Sequence
  Nucleic acid sequence used for crosslinking
aggcgcccaauacgaccaaauc

SEQ ID NO: 139 - RNA, 21 nt, Artificial Sequence
  Nucleic acid sequence used for crosslinking
gauaagaugaaucucuucucc

SEQ ID NO: 140 - RNA, 21 nt, Artificial Sequence
  Nucleic acid sequence used for crosslinking
agaagagauucaucuuaucuc

SEQ ID NO: 141 - RNA, 22 nt, Artificial Sequence
  Nucleic acid sequence used for crosslinking
uuuggucguauugggcgccugg

SEQ ID NO: 142 - RNA, 22 nt, Artificial Sequence
  Nucleic acid sequence used for crosslinking
aggcgcccaauacgaccaaauc

SEQ ID NO: 143 - RNA, 21 nt, Artificial Sequence
  Nucleic acid sequence used for crosslinking
gauaagaugaaucucuucucc

SEQ ID NO: 144 - RNA, 21 nt, Artificial Sequence
  Nucleic acid sequence used for crosslinking
agaagagauucaucuuaucuc

SEQ ID NO: 145 - RNA, 22 nt, Artificial Sequence
  Nucleic acid sequence used for crosslinking
uuuggucguauugggcgccugg

SEQ ID NO: 146 - RNA, 22 nt, Artificial Sequence
  Nucleic acid sequence used for crosslinking
aggcgcccaauacgaccaaauc

SEQ ID NO: 147 - RNA, 22 nt, Artificial Sequence
  Nucleic acid sequence used for crosslinking
agauaagaugaaucucuucucc

SEQ ID NO: 148 - RNA, 20 nt, Artificial Sequence
  Nucleic acid sequence used for crosslinking
agaagagauucaucuuaucu

SEQ ID NO: 149 - RNA, 22 nt, Artificial Sequence
  Nucleic acid sequence used for crosslinking
uuuggucguauugggcgccugg

SEQ ID NO: 150 - RNA, 20 nt, Artificial Sequence
  Nucleic acid sequence used for crosslinking
aggcgcccaauacgaccaaa

SEQ ID NO: 151 - RNA, 22 nt, Artificial Sequence
  Nucleic acid sequence used for crosslinking
agauaagaugaaucucuucucc

SEQ ID NO: 152 - RNA, 21 nt, Artificial Sequence
  Nucleic acid sequence used for crosslinking
agaagagauucaucuuaucuc

SEQ ID NO: 153 - RNA, 22 nt, Artificial Sequence
  Nucleic acid sequence used for crosslinking
uuuggucguauugggcgccugg

SEQ ID NO: 154 - RNA, 21 nt, Artificial Sequence
  Nucleic acid sequence used for crosslinking
aggcgcccaauacgaccaaau

SEQ ID NO: 155 - RNA, 22 nt, Artificial Sequence
  Nucleic acid sequence used for crosslinking
acuuuguuggauuugaaauucc

SEQ ID NO: 156 - RNA, 21 nt, Artificial Sequence
  Nucleic acid sequence used for crosslinking
aauuucaaauccaacaaaguc

SEQ ID NO: 157 - RNA, 22 nt, Artificial Sequence
  Nucleic acid sequence used for crosslinking
agauaagaugaaucucuucucc

SEQ ID NO: 158 - RNA, 23 nt, Artificial Sequence
  Nucleic acid sequence used for crosslinking
agaagagauucaucuuaucucca

SEQ ID NO: 159 - RNA, 22 nt, Artificial Sequence
  Nucleic acid sequence used for crosslinking
uuuggucguauugggcgccugg

SEQ ID NO: 160 - RNA, 23 nt, Artificial Sequence
  Nucleic acid sequence used for crosslinking
aggcgcccaauacgaccaaaucc

SEQ ID NO: 161 - RNA, 22 nt, Artificial Sequence
  Nucleic acid sequence used for crosslinking
agauaagaugaaucucuucucc

SEQ ID NO: 162 - RNA, 23 nt, Artificial Sequence
  Nucleic acid sequence used for crosslinking
agaagagauucaucuuaucucca

SEQ ID NO: 163 - RNA, 22 nt, Artificial Sequence
  Nucleic acid sequence used for crosslinking
uuuggucguauugggcgccugg

SEQ ID NO: 164 - RNA, 23 nt, Artificial Sequence
  Nucleic acid sequence used for crosslinking
aggcgcccaauacgaccaaaucc

SEQ ID NO: 165 - RNA, 22 nt, Artificial Sequence
  Nucleic acid sequence used for crosslinking
agauaagaugaaucucuucucc

SEQ ID NO: 166 - RNA, 23 nt, Artificial Sequence
  Nucleic acid sequence used for crosslinking
agaagagauucaucuuaucucca

SEQ ID NO: 167 - RNA, 22 nt, Artificial Sequence
  Nucleic acid sequence used for crosslinking
acuuuguuggauuugaaauucc

SEQ ID NO: 168 - RNA, 23 nt, Artificial Sequence
  Nucleic acid sequence used for crosslinking
aauuucaaauccaacaaagucug

SEQ ID NO: 169 - RNA, 22 nt, Artificial Sequence
  Nucleic acid sequence used for crosslinking
agauaagaugaaucucuucucc

SEQ ID NO: 170 - RNA, 24 nt, Artificial Sequence
  Nucleic acid sequence used for crosslinking
agaagagauucaucuuaucuccau

SEQ ID NO: 171 - RNA, 22 nt, Artificial Sequence
  Nucleic acid sequence used for crosslinking
uuuggucguauugggcgccugg

SEQ ID NO: 172 - RNA, 24 nt, Artificial Sequence
  Nucleic acid sequence used for crosslinking
aggcgcccaauacgaccaaauccg

SEQ ID NO: 173 - RNA, 22 nt, Artificial Sequence
  Nucleic acid sequence used for crosslinking
agauaagaugaaucucuucucc

SEQ ID NO: 174 - RNA, 24 nt, Artificial Sequence
  Nucleic acid sequence used for crosslinking
agaagagauucaucuuaucuccau

SEQ ID NO: 175 - RNA, 22 nt, Artificial Sequence
  Nucleic acid sequence used for crosslinking
acuuuguuggauuugaaauucc

SEQ ID NO: 176 - RNA, 24 nt, Artificial Sequence
  Nucleic acid sequence used for crosslinking
aauuucaaauccaacaaagucugg

SEQ ID NO: 177 - RNA, 22 nt, Artificial Sequence
  Nucleic acid sequence used for crosslinking
agauaagaugaaucucuucucc

SEQ ID NO: 178 - RNA, 24 nt, Artificial Sequence
  Nucleic acid sequence used for crosslinking
agaagagauucaucuuaucuccau

SEQ ID NO: 179 - RNA, 20 nt, Artificial Sequence
  Nucleic acid sequence used for crosslinking
uuuggucguauugggcgccu

SEQ ID NO: 180 - RNA, 22 nt, Artificial Sequence
  Nucleic acid sequence used for crosslinking
aggcgcccaauacgaccaaauc

SEQ ID NO: 181 - RNA, 20 nt, Artificial Sequence
  Nucleic acid sequence used for crosslinking
acuuuguuggauuugaaauu

SEQ ID NO: 182 - RNA, 22 nt, Artificial Sequence
  Nucleic acid sequence used for crosslinking
aauuucaaauccaacaaagucu

SEQ ID NO: 183 - RNA, 24 nt, Artificial Sequence
  Nucleic acid sequence used for crosslinking
uuuggucguauugggcgccugguc

SEQ ID NO: 184 - RNA, 22 nt, Artificial Sequence
  Nucleic acid sequence used for crosslinking
aggcgcccaauacgaccaaauc

SEQ ID NO: 185 - RNA, 21 nt, Artificial Sequence
  Nucleic acid sequence used for crosslinking
gauaagaugaaucucuucucc

SEQ ID NO: 186 - RNA, 22 nt, Artificial Sequence
  Nucleic acid sequence used for crosslinking
agaagagauucaucuuaucucc

SEQ ID NO: 187 - RNA, 21 nt, Artificial Sequence
  Nucleic acid sequence used for crosslinking
uuggucguauugggcgccugg

SEQ ID NO: 188 - RNA, 22 nt, Artificial Sequence
  Nucleic acid sequence used for crosslinking
aggcgcccaauacgaccaaauc

SEQ ID NO: 189 - RNA, 19 nt, Artificial Sequence
  Nucleic acid sequence used for crosslinking
uaagaugaaucucuucucc

SEQ ID NO: 190 - RNA, 22 nt, Artificial Sequence
  Nucleic acid sequence used for crosslinking
agaagagauucaucuuaucucc

SEQ ID NO: 191 - RNA, 20 nt, Artificial Sequence
  Nucleic acid sequence used for crosslinking
uggucguauugggcgccugg

SEQ ID NO: 192 - RNA, 22 nt, Artificial Sequence
  Nucleic acid sequence used for crosslinking
aggcgcccaauacgaccaaauc

SEQ ID NO: 193 - RNA, 18 nt, Artificial Sequence
  Nucleic acid sequence used for crosslinking
aagaugaaucucuucucc

SEQ ID NO: 194 - RNA, 22 nt, Artificial Sequence
  Nucleic acid sequence used for crosslinking
agaagagauucaucuuaucucc

SEQ ID NO: 195 - RNA, 19 nt, Artificial Sequence
  Nucleic acid sequence used for crosslinking
ggucguauugggcgccugg

SEQ ID NO: 196 - RNA, 22 nt, Artificial Sequence
  Nucleic acid sequence used for crosslinking
aggcgcccaauacgaccaaauc

SEQ ID NO: 197 - RNA, 17 nt, Artificial Sequence
  Nucleic acid sequence used for crosslinking
agaugaaucucuucucc

SEQ ID NO: 198 - RNA, 22 nt, Artificial Sequence
  Nucleic acid sequence used for crosslinking
agaagagauucaucuuaucucc

SEQ ID NO: 199 - RNA, 18 nt, Artificial Sequence
  Nucleic acid sequence used for crosslinking
gucguauugggcgccugg

SEQ ID NO: 200 - RNA, 22 nt, Artificial Sequence
  Nucleic acid sequence used for crosslinking
aggcgcccaauacgaccaaauc

SEQ ID NO: 201 - RNA, 21 nt, Artificial Sequence
  Nucleic acid sequence used for crosslinking
gauaagaugaaucucuucucc

SEQ ID NO: 202 - RNA, 21 nt, Artificial Sequence
  Nucleic acid sequence used for crosslinking
agaagagauucaucuuaucuc

SEQ ID NO: 203 - RNA, 21 nt, Artificial Sequence
  Nucleic acid sequence used for crosslinking
gauaagaugaaucucuucucc

SEQ ID NO: 204 - RNA, 21 nt, Artificial Sequence
  Nucleic acid sequence used for crosslinking
agaagagauucaucuuaucuc

SEQ ID NO: 205 - RNA, 21 nt, Artificial Sequence
  Nucleic acid sequence used for crosslinking
gauaagaugaaucucuucucc

SEQ ID NO: 206 - RNA, 21 nt, Artificial Sequence
  Nucleic acid sequence used for crosslinking
agaagagauucaucuuaucuc

SEQ ID NO: 207 - RNA, 21 nt, Artificial Sequence
  Nucleic acid sequence used for crosslinking
gauaagaugaaucucuucucc

SEQ ID NO: 208 - RNA, 21 nt, Artificial Sequence
  Nucleic acid sequence used for crosslinking
agaagagauucaucuuaucuc

SEQ ID NO: 209 - RNA, 22 nt, Artificial Sequence
  Nucleic acid sequence used for crosslinking
agauaagaugaaucucuucucc

SEQ ID NO: 210 - RNA, 22 nt, Artificial Sequence
  Nucleic acid sequence used for crosslinking
agaagagauucaucuuaucucc

SEQ ID NO: 211 - RNA, 22 nt, Artificial Sequence
  Nucleic acid sequence used for crosslinking
agauaagaugaaucucuucucc

SEQ ID NO: 212 - RNA, 22 nt, Artificial Sequence
  Nucleic acid sequence used for crosslinking
agaagagauucaucuuaucucc

SEQ ID NO: 213 - RNA, 22 nt, Artificial Sequence
  Nucleic acid sequence used for crosslinking
agauaagaugaaucucuucucc

SEQ ID NO: 214 - RNA, 22 nt, Artificial Sequence
  Nucleic acid sequence used for crosslinking
agaagagauucaucuuaucucc

SEQ ID NO: 215 - RNA, 22 nt, Artificial Sequence
  Nucleic acid sequence used for crosslinking
agauaagaugaaucucuucucc

SEQ ID NO: 216 - RNA, 22 nt, Artificial Sequence
  Nucleic acid sequence used for crosslinking
agaagagauucaucuuaucucc

SEQ ID NO: 217 - RNA, 21 nt, Artificial Sequence
  Nucleic acid sequence used for crosslinking
gauaagaugaaucucuucucc

SEQ ID NO: 218 - RNA, 21 nt, Artificial Sequence
  Nucleic acid sequence used for crosslinking
agaagagauucaucuuaucuc

SEQ ID NO: 219 - RNA, 22 nt, Artificial Sequence
  Nucleic acid sequence used for crosslinking
uuuggucguauugggcgccugg

SEQ ID NO: 220 - RNA, 22 nt, Artificial Sequence
  Nucleic acid sequence used for crosslinking
aggcgcccaauacgaccaaauc

SEQ ID NO: 221 - RNA, 21 nt, Artificial Sequence
  Nucleic acid sequence used for crosslinking
gauaagaugaaucucuucucc

SEQ ID NO: 222 - RNA, 21 nt, Artificial Sequence
  Nucleic acid sequence used for crosslinking
agaagagauucaucuuaucuc

SEQ ID NO: 223 - RNA, 22 nt, Artificial Sequence
  Nucleic acid sequence used for crosslinking
uuuggucguauugggcgccugg

SEQ ID NO: 224 - RNA, 22 nt, Artificial Sequence
  Nucleic acid sequence used for crosslinking
aggcgcccaauacgaccaaauc

SEQ ID NO: 225 - RNA, 21 nt, Artificial Sequence
  Nucleic acid sequence used for crosslinking
gauaagaugaaucucuucucc

SEQ ID NO: 226 - RNA, 21 nt, Artificial Sequence
  Nucleic acid sequence used for crosslinking
agaagagauucaucuuaucuc

SEQ ID NO: 227 - RNA, 22 nt, Artificial Sequence
  Nucleic acid sequence used for crosslinking
uuuggucguauugggcgccugg

SEQ ID NO: 228 - RNA, 22 nt, Artificial Sequence
  Nucleic acid sequence used for crosslinking
aggcgcccaauacgaccaaauc

SEQ ID NO: 229 - RNA, 21 nt, Artificial Sequence
  Nucleic acid sequence used for crosslinking
gauaagaugaaucucuucucc

SEQ ID NO: 230 - RNA, 21 nt, Artificial Sequence
  Nucleic acid sequence used for crosslinking
agaagagauucaucuuaucuc

SEQ ID NO: 231 - RNA, 22 nt, Artificial Sequence
  Nucleic acid sequence used for crosslinking
uuuggucguauugggcgccugg

SEQ ID NO: 232 - RNA, 22 nt, Artificial Sequence
  Nucleic acid sequence used for crosslinking
aggcgcccaauacgaccaaauc

SEQ ID NO: 233 - RNA, 21 nt, Artificial Sequence
  Nucleic acid sequence used for crosslinking
gauaagaugaaucucuucucc

SEQ ID NO: 234 - RNA, 21 nt, Artificial Sequence
  Nucleic acid sequence used for crosslinking
agaagagauucaucuuaucuc

SEQ ID NO: 235 - RNA, 21 nt, Artificial Sequence
  Nucleic acid sequence used for crosslinking
gauaagaugaaucucuucucc

SEQ ID NO: 236 - RNA, 21 nt, Artificial Sequence
  Nucleic acid sequence used for crosslinking
agaagagauucaucuuaucuc

SEQ ID NO: 237 - RNA, 22 nt, Artificial Sequence
  Nucleic acid sequence used for crosslinking
uuuggucguauugggcgccugg

SEQ ID NO: 238 - RNA, 22 nt, Artificial Sequence
  Nucleic acid sequence used for crosslinking
aggcgcccaauacgaccaaauc

SEQ ID NO: 239 - RNA, 21 nt, Artificial Sequence
  Nucleic acid sequence used for crosslinking
gauaagaugaaucucuucucc

SEQ ID NO: 240 - RNA, 21 nt, Artificial Sequence
  Nucleic acid sequence used for crosslinking
agaagagauucaucuuaucuc

SEQ ID NO: 241 - RNA, 22 nt, Artificial Sequence
  Nucleic acid sequence used for crosslinking
uuuggucguauugggcgccugg

SEQ ID NO: 242 - RNA, 22 nt, Artificial Sequence
  Nucleic acid sequence used for crosslinking
aggcgcccaauacgaccaaauc

SEQ ID NO: 243 - RNA, 21 nt, Artificial Sequence
  Nucleic acid sequence used for crosslinking
gauaagaugaaucucuucucc

SEQ ID NO: 244 - RNA, 21 nt, Artificial Sequence
  Nucleic acid sequence used for crosslinking
agaagagauucaucuuaucuc

SEQ ID NO: 245 - RNA, 22 nt, Artificial Sequence
  Nucleic acid sequence used for crosslinking
uuuggucguauugggcgccugg

SEQ ID NO: 246 - RNA, 22 nt, Artificial Sequence
  Nucleic acid sequence used for crosslinking
aggcgcccaauacgaccaaauc

SEQ ID NO: 247 - RNA, 21 nt, Artificial Sequence
  Nucleic acid sequence used for crosslinking
gauaagaugaaucucuucucc

SEQ ID NO: 248 - RNA, 21 nt, Artificial Sequence
  Nucleic acid sequence used for crosslinking
agaagagauucaucuuaucuc

SEQ ID NO: 249 - RNA, 22 nt, Artificial Sequence
  Nucleic acid sequence used for crosslinking
uuuggucguauugggcgccugg

SEQ ID NO: 250 - RNA, 22 nt, Artificial Sequence
  Nucleic acid sequence used for crosslinking
aggcgcccaauacgaccaaauc

SEQ ID NO: 251 - RNA, 21 nt, Artificial Sequence
  Nucleic acid sequence used for crosslinking
gauaagaugaaucucuucucc

SEQ ID NO: 252 - RNA, 21 nt, Artificial Sequence
  Nucleic acid sequence used for crosslinking
agaagagauucaucuuaucuc

SEQ ID NO: 253 - RNA, 22 nt, Artificial Sequence
  Nucleic acid sequence used for crosslinking
uuuggucguauugggcgccugg

SEQ ID NO: 254 - RNA, 22 nt, Artificial Sequence
  Nucleic acid sequence used for crosslinking
aggcgcccaauacgaccaaauc

SEQ ID NO: 255 - RNA, 21 nt, Artificial Sequence
  Nucleic acid sequence used for crosslinking
gauaagaugaaucucuucucc

SEQ ID NO: 256 - RNA, 21 nt, Artificial Sequence
  Nucleic acid sequence used for crosslinking
agaagagauucaucuuaucuc

SEQ ID NO: 257 - RNA, 22 nt, Artificial Sequence
  Nucleic acid sequence used for crosslinking
uuuggucguauugggcgccugg

SEQ ID NO: 258 - RNA, 22 nt, Artificial Sequence
  Nucleic acid sequence used for crosslinking
aggcgcccaauacgaccaaauc

SEQ ID NO: 259 - RNA, 21 nt, Artificial Sequence
  Nucleic acid sequence used for crosslinking
gauaagaugaaucucuucucc

SEQ ID NO: 260 - RNA, 21 nt, Artificial Sequence
  Nucleic acid sequence used for crosslinking
agaagagauucaucuuaucuc

SEQ ID NO: 261 - RNA, 22 nt, Artificial Sequence
  Nucleic acid sequence used for crosslinking
uuuggucguauugggcgccugg

SEQ ID NO: 262 - RNA, 22 nt, Artificial Sequence
  Nucleic acid sequence used for crosslinking
aggcgcccaauacgaccaaauc

SEQ ID NO: 263 - RNA, 21 nt, Artificial Sequence
  Nucleic acid sequence used for crosslinking
gauaagaugaaucucuucucc

SEQ ID NO: 264 - RNA, 21 nt, Artificial Sequence
  Nucleic acid sequence used for crosslinking
agaagagauucaucuuaucuc

SEQ ID NO: 265 - RNA, 22 nt, Artificial Sequence
  Nucleic acid sequence used for crosslinking
uuuggucguauugggcgccugg

SEQ ID NO: 266 - RNA, 22 nt, Artificial Sequence
  Nucleic acid sequence used for crosslinking
aggcgcccaauacgaccaaauc

SEQ ID NO: 267 - RNA, 21 nt, Artificial Sequence
  Nucleic acid sequence used for crosslinking
gauaagaugaaucucuucucc

SEQ ID NO: 268 - RNA, 21 nt, Artificial Sequence
  Nucleic acid sequence used for crosslinking
agaagagauucaucuuaucuc

SEQ ID NO: 269 - RNA, 22 nt, Artificial Sequence
  Nucleic acid sequence used for crosslinking
uuuggucguauugggcgccugg

SEQ ID NO: 270 - RNA, 22 nt, Artificial Sequence
  Nucleic acid sequence used for crosslinking
aggcgcccaauacgaccaaauc

SEQ ID NO: 271 - RNA, 21 nt, Artificial Sequence
  Nucleic acid sequence used for crosslinking
gauaagaugaaucucuucucc

SEQ ID NO: 272 - RNA, 21 nt, Artificial Sequence
  Nucleic acid sequence used for crosslinking
agaagagauucaucuuaucuc

SEQ ID NO: 273 - RNA, 21 nt, Artificial Sequence
  Nucleic acid sequence used for crosslinking
gauaagaugaaucucuucucc

SEQ ID NO: 274 - RNA, 21 nt, Artificial Sequence
  Nucleic acid sequence used for crosslinking
agaagagauucaucuuaucuc

SEQ ID NO: 275 - RNA, 22 nt, Artificial Sequence
  Nucleic acid sequence used for crosslinking
uuuggucguauugggcgccugg

SEQ ID NO: 276 - RNA, 22 nt, Artificial Sequence
  Nucleic acid sequence used for crosslinking
aggcgcccaauacgaccaaauc

SEQ ID NO: 277 - RNA, 21 nt, Artificial Sequence
  Nucleic acid sequence used for crosslinking
gauaagaugaaucucuucucc

SEQ ID NO: 278 - RNA, 21 nt, Artificial Sequence
  Nucleic acid sequence used for crosslinking
agaagagauucaucuuaucuc

SEQ ID NO: 279 - RNA, 22 nt, Artificial Sequence
  Nucleic acid sequence used for crosslinking
uuuggucguauugggcgccugg

SEQ ID NO: 280 - RNA, 22 nt, Artificial Sequence
  Nucleic acid sequence used for crosslinking
aggcgcccaauacgaccaaauc

SEQ ID NO: 281 - RNA, 21 nt, Artificial Sequence
  Nucleic acid sequence used for crosslinking
gauaagaugaaucucuucucc

SEQ ID NO: 282 - RNA, 21 nt, Artificial Sequence
  Nucleic acid sequence used for crosslinking
agaagagauucaucuuaucuc

SEQ ID NO: 283 - RNA, 22 nt, Artificial Sequence
  Nucleic acid sequence used for crosslinking
uuuggucguauugggcgccugg

SEQ ID NO: 284 - RNA, 22 nt, Artificial Sequence
  Nucleic acid sequence used for crosslinking
aggcgcccaauacgaccaaauc

SEQ ID NO: 285 - RNA, 22 nt, Artificial Sequence
  Nucleic acid sequence used for crosslinking
uuuggucguauugggcgccugg

SEQ ID NO: 286 - RNA, 22 nt, Artificial Sequence
  Nucleic acid sequence used for crosslinking
aggcgcccaauacgaccaaauc

SEQ ID NO: 287 - RNA, 22 nt, Artificial Sequence
  Nucleic acid sequence used for crosslinking
uuuggucguauugggcgccugg

SEQ ID NO: 288 - RNA, 22 nt, Artificial Sequence
  Nucleic acid sequence used for crosslinking
aggcgcccaauacgaccaaauc

SEQ ID NO: 289 - RNA, 22 nt, Artificial Sequence
  Nucleic acid sequence used for crosslinking
uuuggucguauugggcgccugg

SEQ ID NO: 290 - RNA, 22 nt, Artificial Sequence
  Nucleic acid sequence used for crosslinking
aggcgcccaauacgaccaaauc

SEQ ID NO: 291 - RNA, 21 nt, Artificial Sequence
  Nucleic acid sequence used for crosslinking
gauaagaugaaucucuucucc

SEQ ID NO: 292 - RNA, 21 nt, Artificial Sequence
  Nucleic acid sequence used for crosslinking
agaagagauucaucuuaucuc

SEQ ID NO: 293 - RNA, 22 nt, Artificial Sequence
  Nucleic acid sequence used for crosslinking
uuuggucguauugggcgccugg

SEQ ID NO: 294 - RNA, 22 nt, Artificial Sequence
  Nucleic acid sequence used for crosslinking
aggcgcccaauacgaccaaauc

SEQ ID NO: 295 - RNA, 22 nt, Artificial Sequence
  Nucleic acid sequence used for crosslinking
uuuggucguauugggcgccugg

SEQ ID NO: 296 - RNA, 22 nt, Artificial Sequence
  Nucleic acid sequence used for crosslinking
aggcgcccaauacgaccaaauc

SEQ ID NO: 297 - RNA, 22 nt, Artificial Sequence
  Nucleic acid sequence used for crosslinking
uuuggucguauugggcgccugg

SEQ ID NO: 298 - RNA, 22 nt, Artificial Sequence
  Nucleic acid sequence used for crosslinking
aggcgcccaauacgaccaaauc

SEQ ID NO: 299 - RNA, 21 nt, Artificial Sequence
  Nucleic acid sequence used for crosslinking
gauaagaugaaucucuucucc

SEQ ID NO: 300 - RNA, 21 nt, Artificial Sequence
  Nucleic acid sequence used for crosslinking
agaagagauucaucuuaucuc

SEQ ID NO: 301 - RNA, 22 nt, Artificial Sequence
  Nucleic acid sequence used for crosslinking
uuuggucguauugggcgccugg

SEQ ID NO: 302 - RNA, 22 nt, Artificial Sequence
  Nucleic acid sequence used for crosslinking
aggcgcccaauacgaccaaauc

SEQ ID NO: 303 - RNA, 22 nt, Artificial Sequence
  Nucleic acid sequence used for crosslinking
acuuuguuggauuugaaauucc

SEQ ID NO: 304 - RNA, 22 nt, Artificial Sequence
  Nucleic acid sequence used for crosslinking
aauuucaaauccaacaaagucu

SEQ ID NO: 305 - RNA, 21 nt, Artificial Sequence
  Nucleic acid sequence used for crosslinking
gauaagaugaaucucuucucc

SEQ ID NO: 306 - RNA, 21 nt, Artificial Sequence
  Nucleic acid sequence used for crosslinking
agaagagauucaucuuaucuc

SEQ ID NO: 307 - RNA, 22 nt, Artificial Sequence
  Nucleic acid sequence used for crosslinking
uuuggucguauugggcgccugg

SEQ ID NO: 308 - RNA, 22 nt, Artificial Sequence
  Nucleic acid sequence used for crosslinking
aggcgcccaauacgaccaaauc

SEQ ID NO: 309 - RNA, 22 nt, Artificial Sequence
  Nucleic acid sequence used for crosslinking
acuuuguuggauuugaaauucc

SEQ ID NO: 310 - RNA, 22 nt, Artificial Sequence
  Nucleic acid sequence used for crosslinking
aauuucaaauccaacaaagucu

SEQ ID NO: 311 - RNA, 21 nt, Artificial Sequence
  Nucleic acid sequence used for crosslinking
gauaagaugaaucucuucucc

SEQ ID NO: 312 - RNA, 21 nt, Artificial Sequence
  Nucleic acid sequence used for crosslinking
agaagagauucaucuuaucuc

SEQ ID NO: 313 - RNA, 22 nt, Artificial Sequence
  Nucleic acid sequence used for crosslinking
uuuggucguauugggcgccugg

SEQ ID NO: 314 - RNA, 22 nt, Artificial Sequence
  Nucleic acid sequence used for crosslinking
aggcgcccaauacgaccaaauc

SEQ ID NO: 315 - RNA, 22 nt, Artificial Sequence
  Nucleic acid sequence used for crosslinking
acuuuguuggauuugaaauucc

SEQ ID NO: 316 - RNA, 22 nt, Artificial Sequence
  Nucleic acid sequence used for crosslinking
aauuucaaauccaacaaagucu

SEQ ID NO: 317 - RNA, 21 nt, Artificial Sequence
  Nucleic acid sequence used for crosslinking
gauaagaugaaucucuucucc

SEQ ID NO: 318 - RNA, 21 nt, Artificial Sequence
  Nucleic acid sequence used for crosslinking
agaagagauucaucuuaucuc

SEQ ID NO: 319 - RNA, 22 nt, Artificial Sequence
  Nucleic acid sequence used for crosslinking
uuuggucguauugggcgccugg

SEQ ID NO: 320 - RNA, 22 nt, Artificial Sequence
  Nucleic acid sequence used for crosslinking
aggcgcccaauacgaccaaauc

SEQ ID NO: 321 - RNA, 22 nt, Artificial Sequence
  Nucleic acid sequence used for crosslinking
acuuuguuggauuugaaauucc

SEQ ID NO: 322 - RNA, 22 nt, Artificial Sequence
  Nucleic acid sequence used for crosslinking
aauuucaaauccaacaaagucu

SEQ ID NO: 323 - RNA, 21 nt, Artificial Sequence
  Nucleic acid sequence used for crosslinking
gauaagaugaaucucuucucc

SEQ ID NO: 324 - RNA, 21 nt, Artificial Sequence
  Nucleic acid sequence used for crosslinking
agaagagauucaucuuaucuc

SEQ ID NO: 325 - RNA, 22 nt, Artificial Sequence
  Nucleic acid sequence used for crosslinking
uuuggucguauugggcgccugg

SEQ ID NO: 326 - RNA, 22 nt, Artificial Sequence
  Nucleic acid sequence used for crosslinking
aggcgcccaauacgaccaaauc

SEQ ID NO: 327 - RNA, 22 nt, Artificial Sequence
  Nucleic acid sequence used for crosslinking
acuuuguuggauuugaaauucc

SEQ ID NO: 328 - RNA, 22 nt, Artificial Sequence
  Nucleic acid sequence used for crosslinking
aauuucaaauccaacaaagucu

SEQ ID NO: 329 - RNA, 21 nt, Artificial Sequence
  Nucleic acid sequence used for crosslinking
gauaagaugaaucucuucucc

SEQ ID NO: 330 - RNA, 21 nt, Artificial Sequence
  Nucleic acid sequence used for crosslinking
agaagagauucaucuuaucuc

SEQ ID NO: 331 - RNA, 22 nt, Artificial Sequence
  Nucleic acid sequence used for crosslinking
uuuggucguauugggcgccugg

SEQ ID NO: 332 - RNA, 22 nt, Artificial Sequence
  Nucleic acid sequence used for crosslinking
aggcgcccaauacgaccaaauc

SEQ ID NO: 333 - RNA, 22 nt, Artificial Sequence
  Nucleic acid sequence used for crosslinking
acuuuguuggauuugaaauucc

SEQ ID NO: 334 - RNA, 22 nt, Artificial Sequence
  Nucleic acid sequence used for crosslinking
aauuucaaauccaacaaagucu

SEQ ID NO: 335 - RNA, 21 nt, Artificial Sequence
  Nucleic acid sequence used for crosslinking
gauaagaugaaucucuucucc

SEQ ID NO: 336 - RNA, 21 nt, Artificial Sequence
  Nucleic acid sequence used for crosslinking
agaagagauucaucuuaucuc

SEQ ID NO: 337 - RNA, 22 nt, Artificial Sequence
  Nucleic acid sequence used for crosslinking
uuuggucguauugggcgccugg

SEQ ID NO: 338 - RNA, 22 nt, Artificial Sequence
  Nucleic acid sequence used for crosslinking
aggcgcccaauacgaccaaauc

SEQ ID NO: 339 - RNA, 22 nt, Artificial Sequence
  Nucleic acid sequence used for crosslinking
acuuuguuggauuugaaauucc

SEQ ID NO: 340 - RNA, 22 nt, Artificial Sequence
  Nucleic acid sequence used for crosslinking
aauuucaaauccaacaaagucu

SEQ ID NO: 341 - RNA, 21 nt, Artificial Sequence
  Nucleic acid sequence used for crosslinking
gauaagaugaaucucuucucc

SEQ ID NO: 342 - RNA, 21 nt, Artificial Sequence
  Nucleic acid sequence used for crosslinking
agaagagauucaucuuaucuc

SEQ ID NO: 343 - RNA, 22 nt, Artificial Sequence
  Nucleic acid sequence used for crosslinking
uuuggucguauugggcgccugg

SEQ ID NO: 344 - RNA, 22 nt, Artificial Sequence
  Nucleic acid sequence used for crosslinking
aggcgcccaauacgaccaaauc

SEQ ID NO: 345 - RNA, 22 nt, Artificial Sequence
  Nucleic acid sequence used for crosslinking
acuuuguuggauuugaaauucc

SEQ ID NO: 346 - RNA, 22 nt, Artificial Sequence
  Nucleic acid sequence used for crosslinking
aauuucaaauccaacaaagucu

SEQ ID NO: 347 - RNA, 21 nt, Artificial Sequence
  Nucleic acid sequence used for crosslinking
gauaagaugaaucucuucucc

SEQ ID NO: 348 - RNA, 21 nt, Artificial Sequence
  Nucleic acid sequence used for crosslinking
agaagagauucaucuuaucuc

SEQ ID NO: 349 - RNA, 22 nt, Artificial Sequence
  Nucleic acid sequence used for crosslinking
uuuggucguauugggcgccugg

SEQ ID NO: 350 - RNA, 22 nt, Artificial Sequence
  Nucleic acid sequence used for crosslinking
aggcgcccaauacgaccaaauc

SEQ ID NO: 351 - RNA, 22 nt, Artificial Sequence
  Nucleic acid sequence used for crosslinking
acuuuguuggauuugaaauucc

SEQ ID NO: 352 - RNA, 22 nt, Artificial Sequence
  Nucleic acid sequence used for crosslinking
aauuucaaauccaacaaagucu

SEQ ID NO: 353 - RNA, 21 nt, Artificial Sequence
  Nucleic acid sequence used for crosslinking
gauaagaugaaucucuucucc

SEQ ID NO: 354 - RNA, 21 nt, Artificial Sequence
  Nucleic acid sequence used for crosslinking
agaagagauucaucuuaucuc

SEQ ID NO: 355 - RNA, 22 nt, Artificial Sequence
  Nucleic acid sequence used for crosslinking
uuuggucguauugggcgccugg

SEQ ID NO: 356 - RNA, 22 nt, Artificial Sequence
  Nucleic acid sequence used for crosslinking
aggcgcccaauacgaccaaauc

SEQ ID NO: 357 - RNA, 22 nt, Artificial Sequence
  Nucleic acid sequence used for crosslinking
acuuuguuggauuugaaauucc

SEQ ID NO: 358 - RNA, 22 nt, Artificial Sequence
  Nucleic acid sequence used for crosslinking
aauuucaaauccaacaaagucu

SEQ ID NO: 359 - RNA, 21 nt, Artificial Sequence
  Nucleic acid sequence used for crosslinking
gauaagaugaaucucuucucc

SEQ ID NO: 360 - RNA, 21 nt, Artificial Sequence
  Nucleic acid sequence used for crosslinking
agaagagauucaucuuaucuc

SEQ ID NO: 361 - RNA, 22 nt, Artificial Sequence
  Nucleic acid sequence used for crosslinking
uuuggucguauugggcgccugg

SEQ ID NO: 362 - RNA, 22 nt, Artificial Sequence
  Nucleic acid sequence used for crosslinking
aggcgcccaauacgaccaaauc

SEQ ID NO: 363 - RNA, 22 nt, Artificial Sequence
  Nucleic acid sequence used for crosslinking
acuuuguuggauuugaaauucc

SEQ ID NO: 364 - RNA, 22 nt, Artificial Sequence
  Nucleic acid sequence used for crosslinking
aauuucaaauccaacaaagucu

SEQ ID NO: 365 - RNA, 21 nt, Artificial Sequence
  Nucleic acid sequence used for crosslinking
gauaagaugaaucucuucucc

SEQ ID NO: 366 - RNA, 21 nt, Artificial Sequence
  Nucleic acid sequence used for crosslinking
agaagagauucaucuuaucuc

SEQ ID NO: 367 - RNA, 22 nt, Artificial Sequence
  Nucleic acid sequence used for crosslinking
uuuggucguauugggcgccugg

SEQ ID NO: 368 - RNA, 22 nt, Artificial Sequence
  Nucleic acid sequence used for crosslinking
aggcgcccaauacgaccaaauc

SEQ ID NO: 369 - RNA, 22 nt, Artificial Sequence
  Nucleic acid sequence used for crosslinking
acuuuguuggauuugaaauucc

SEQ ID NO: 370 - RNA, 22 nt, Artificial Sequence
  Nucleic acid sequence used for crosslinking
aauuucaaauccaacaaagucu

SEQ ID NO: 371 - RNA, 21 nt, Artificial Sequence
  Nucleic acid sequence used for crosslinking
gauaagaugaaucucuucucc

SEQ ID NO: 372 - RNA, 21 nt, Artificial Sequence
  Nucleic acid sequence used for crosslinking
agaagagauucaucuuaucuc

SEQ ID NO: 373 - RNA, 22 nt, Artificial Sequence
  Nucleic acid sequence used for crosslinking
uuuggucguauugggcgccugg

SEQ ID NO: 374 - RNA, 22 nt, Artificial Sequence
  Nucleic acid sequence used for crosslinking
aggcgcccaauacgaccaaauc

SEQ ID NO: 375 - RNA, 22 nt, Artificial Sequence
  Nucleic acid sequence used for crosslinking
acuuuguuggauuugaaauucc

SEQ ID NO: 376 - RNA, 22 nt, Artificial Sequence
  Nucleic acid sequence used for crosslinking
aauuucaaauccaacaaagucu

SEQ ID NO: 377 - RNA, 21 nt, Artificial Sequence
  Nucleic acid sequence used for crosslinking
gauaagaugaaucucuucucc

SEQ ID NO: 378 - RNA, 21 nt, Artificial Sequence
  Nucleic acid sequence used for crosslinking
agaagagauucaucuuaucuc

SEQ ID NO: 379 - RNA, 22 nt, Artificial Sequence
  Nucleic acid sequence used for crosslinking
uuuggucguauugggcgccugg

SEQ ID NO: 380 - RNA, 22 nt, Artificial Sequence
  Nucleic acid sequence used for crosslinking
aggcgcccaauacgaccaaauc

SEQ ID NO: 381 - RNA, 22 nt, Artificial Sequence
  Nucleic acid sequence used for crosslinking
acuuuguuggauuugaaauucc

SEQ ID NO: 382 - RNA, 22 nt, Artificial Sequence
  Nucleic acid sequence used for crosslinking
aauuucaaauccaacaaagucu

SEQ ID NO: 383 - RNA, 21 nt, Artificial Sequence
  Nucleic acid sequence used for crosslinking
gauaagaugaaucucuucucc

SEQ ID NO: 384 - RNA, 21 nt, Artificial Sequence
  Nucleic acid sequence used for crosslinking
agaagagauucaucuuaucuc

SEQ ID NO: 385 - RNA, 22 nt, Artificial Sequence
  Nucleic acid sequence used for crosslinking
uuuggucguauugggcgccugg

SEQ ID NO: 386 - RNA, 22 nt, Artificial Sequence
  Nucleic acid sequence used for crosslinking
aggcgcccaauacgaccaaauc

SEQ ID NO: 387 - RNA, 22 nt, Artificial Sequence
  Nucleic acid sequence used for crosslinking
acuuuguuggauuugaaauucc

SEQ ID NO: 388 - RNA, 22 nt, Artificial Sequence
  Nucleic acid sequence used for crosslinking
aauuucaaauccaacaaagucu

SEQ ID NO: 389 - RNA, 21 nt, Artificial Sequence
  Nucleic acid sequence used for crosslinking
gauaagaugaaucucuucucc

SEQ ID NO: 390 - RNA, 21 nt, Artificial Sequence
  Nucleic acid sequence used for crosslinking
agaagagauucaucuuaucuc

SEQ ID NO: 391 - RNA, 22 nt, Artificial Sequence
  Nucleic acid sequence used for crosslinking
uuuggucguauugggcgccugg

SEQ ID NO: 392 - RNA, 22 nt, Artificial Sequence
  Nucleic acid sequence used for crosslinking
aggcgcccaauacgaccaaauc

SEQ ID NO: 393 - RNA, 22 nt, Artificial Sequence
  Nucleic acid sequence used for crosslinking
acuuuguuggauuugaaauucc

SEQ ID NO: 394 - RNA, 22 nt, Artificial Sequence
  Nucleic acid sequence used for crosslinking
aauuucaaauccaacaaagucu

SEQ ID NO: 395 - RNA, 21 nt, Artificial Sequence
  Nucleic acid sequence used for crosslinking
gauaagaugaaucucuucucc

SEQ ID NO: 396 - RNA, 21 nt, Artificial Sequence
  Nucleic acid sequence used for crosslinking
agaagagauucaucuuaucuc

SEQ ID NO: 397 - RNA, 22 nt, Artificial Sequence
  Nucleic acid sequence used for crosslinking
uuuggucguauugggcgccugg

SEQ ID NO: 398 - RNA, 22 nt, Artificial Sequence
  Nucleic acid sequence used for crosslinking
aggcgcccaauacgaccaaauc

SEQ ID NO: 399 - RNA, 22 nt, Artificial Sequence
  Nucleic acid sequence used for crosslinking
acuuuguuggauuugaaauucc

SEQ ID NO: 400 - RNA, 22 nt, Artificial Sequence
  Nucleic acid sequence used for crosslinking
aauuucaaauccaacaaagucu

SEQ ID NO: 401 - RNA, 21 nt, Artificial Sequence
  Nucleic acid sequence used for crosslinking
gauaagaugaaucucuucucc

SEQ ID NO: 402 - RNA, 21 nt, Artificial Sequence
  Nucleic acid sequence used for crosslinking
agaagagauucaucuuaucuc

SEQ ID NO: 403 - RNA, 22 nt, Artificial Sequence
  Nucleic acid sequence used for crosslinking
uuuggucguauugggcgccugg

SEQ ID NO: 404 - RNA, 22 nt, Artificial Sequence
  Nucleic acid sequence used for crosslinking
aggcgcccaauacgaccaaauc

SEQ ID NO: 405 - RNA, 22 nt, Artificial Sequence
  Nucleic acid sequence used for crosslinking
acuuuguuggauuugaaauucc

SEQ ID NO: 406 - RNA, 22 nt, Artificial Sequence
  Nucleic acid sequence used for crosslinking
aauuucaaauccaacaaagucu

SEQ ID NO: 407 - RNA, 21 nt, Artificial Sequence
  Nucleic acid sequence used for crosslinking
gauaagaugaaucucuucucc

SEQ ID NO: 408 - RNA, 21 nt, Artificial Sequence
  Nucleic acid sequence used for crosslinking
agaagagauucaucuuaucuc

SEQ ID NO: 409 - RNA, 22 nt, Artificial Sequence
  Nucleic acid sequence used for crosslinking
uuuggucguauugggcgccugg

SEQ ID NO: 410 - RNA, 22 nt, Artificial Sequence
  Nucleic acid sequence used for crosslinking
aggcgcccaauacgaccaaauc

SEQ ID NO: 411 - RNA, 22 nt, Artificial Sequence
  Nucleic acid sequence used for crosslinking
acuuuguuggauuugaaauucc

SEQ ID NO: 412 - RNA, 22 nt, Artificial Sequence
  Nucleic acid sequence used for crosslinking
aauuucaaauccaacaaagucu

SEQ ID NO: 413 - RNA, 21 nt, Artificial Sequence
  Nucleic acid sequence used for crosslinking
gauaagaugaaucucuucucc

SEQ ID NO: 414 - RNA, 21 nt, Artificial Sequence
  Nucleic acid sequence used for crosslinking
agaagagauucaucuuaucuc

SEQ ID NO: 415 - RNA, 22 nt, Artificial Sequence
  Nucleic acid sequence used for crosslinking
uuuggucguauugggcgccugg

SEQ ID NO: 416 - RNA, 22 nt, Artificial Sequence
  Nucleic acid sequence used for crosslinking
aggcgcccaauacgaccaaauc

SEQ ID NO: 417 - RNA, 22 nt, Artificial Sequence
  Nucleic acid sequence used for crosslinking
acuuuguuggauuugaaauucc

SEQ ID NO: 418 - RNA, 22 nt, Artificial Sequence
  Nucleic acid sequence used for crosslinking
aauuucaaauccaacaaagucu

SEQ ID NO: 419 - RNA, 21 nt, Artificial Sequence
  Nucleic acid sequence used for crosslinking
gauaagaugaaucucuucucc

SEQ ID NO: 420 - RNA, 21 nt, Artificial Sequence
  Nucleic acid sequence used for crosslinking
agaagagauucaucuuaucuc

SEQ ID NO: 421 - RNA, 22 nt, Artificial Sequence
  Nucleic acid sequence used for crosslinking
uuuggucguauugggcgccugg

SEQ ID NO: 422 - RNA, 22 nt, Artificial Sequence
  Nucleic acid sequence used for crosslinking
aggcgcccaauacgaccaaauc

SEQ ID NO: 423 - RNA, 22 nt, Artificial Sequence
  Nucleic acid sequence used for crosslinking
acuuuguuggauuugaaauucc

SEQ ID NO: 424 - RNA, 22 nt, Artificial Sequence
  Nucleic acid sequence used for crosslinking
aauuucaaauccaacaaagucu

SEQ ID NO: 425 - RNA, 21 nt, Artificial Sequence
  Nucleic acid sequence used for crosslinking
gauaagaugaaucucuucucc

SEQ ID NO: 426 - RNA, 21 nt, Artificial Sequence
  Nucleic acid sequence used for crosslinking
agaagagauucaucuuaucuc

SEQ ID NO: 427 - RNA, 22 nt, Artificial Sequence
  Nucleic acid sequence used for crosslinking
uuuggucguauugggcgccugg

SEQ ID NO: 428 - RNA, 22 nt, Artificial Sequence
  Nucleic acid sequence used for crosslinking
aggcgcccaauacgaccaaauc

SEQ ID NO: 429 - RNA, 22 nt, Artificial Sequence
  Nucleic acid sequence used for crosslinking
acuuuguuggauuugaaauucc

SEQ ID NO: 430 - RNA, 22 nt, Artificial Sequence
  Nucleic acid sequence used for crosslinking
aauuucaaauccaacaaagucu

SEQ ID NO: 431 - RNA, 21 nt, Artificial Sequence
  Nucleic acid sequence used for crosslinking
gauaagaugaaucucuucucc

SEQ ID NO: 432 - RNA, 21 nt, Artificial Sequence
  Nucleic acid sequence used for crosslinking
agaagagauucaucuuaucuc

SEQ ID NO: 433 - RNA, 22 nt, Artificial Sequence
  Nucleic acid sequence used for crosslinking
uuuggucguauugggcgccugg

SEQ ID NO: 434 - RNA, 22 nt, Artificial Sequence
  Nucleic acid sequence used for crosslinking
aggcgcccaauacgaccaaauc

SEQ ID NO: 435 - RNA, 22 nt, Artificial Sequence
  Nucleic acid sequence used for crosslinking
acuuuguuggauuugaaauucc

SEQ ID NO: 436 - RNA, 22 nt, Artificial Sequence
  Nucleic acid sequence used for crosslinking
aauuucaaauccaacaaagucu

SEQ ID NO: 437 - RNA, 21 nt, Artificial Sequence
  Nucleic acid sequence used for crosslinking
gauaagaugaaucucuucucc

SEQ ID NO: 438 - RNA, 21 nt, Artificial Sequence
  Nucleic acid sequence used for crosslinking
agaagagauucaucuuaucuc

SEQ ID NO: 439 - RNA, 22 nt, Artificial Sequence
  Nucleic acid sequence used for crosslinking
uuuggucguauugggcgccugg

SEQ ID NO: 440 - RNA, 22 nt, Artificial Sequence
  Nucleic acid sequence used for crosslinking
aggcgcccaauacgaccaaauc

SEQ ID NO: 441 - RNA, 22 nt, Artificial Sequence
  Nucleic acid sequence used for crosslinking
acuuuguuggauuugaaauucc

SEQ ID NO: 442 - RNA, 22 nt, Artificial Sequence
  Nucleic acid sequence used for crosslinking
aauuucaaauccaacaaagucu

SEQ ID NO: 443 - RNA, 21 nt, Artificial Sequence
  Nucleic acid sequence used for crosslinking
gauaagaugaaucucuucucc

SEQ ID NO: 444 - RNA, 21 nt, Artificial Sequence
  Nucleic acid sequence used for crosslinking
agaagagauucaucuuaucuc

SEQ ID NO: 445 - RNA, 22 nt, Artificial Sequence
  Nucleic acid sequence used for crosslinking
uuuggucguauugggcgccugg

SEQ ID NO: 446 - RNA, 22 nt, Artificial Sequence
  Nucleic acid sequence used for crosslinking
aggcgcccaauacgaccaaauc

SEQ ID NO: 447 - RNA, 22 nt, Artificial Sequence
  Nucleic acid sequence used for crosslinking
acuuuguuggauuugaaauucc

SEQ ID NO: 448 - RNA, 22 nt, Artificial Sequence
  Nucleic acid sequence used for crosslinking
aauuucaaauccaacaaagucu

SEQ ID NO: 449 - RNA, 21 nt, Artificial Sequence
  Nucleic acid sequence used for crosslinking
gauaagaugaaucucuucucc

SEQ ID NO: 450 - RNA, 21 nt, Artificial Sequence
  Nucleic acid sequence used for crosslinking
agaagagauucaucuuaucuc

SEQ ID NO: 451 - RNA, 22 nt, Artificial Sequence
  Nucleic acid sequence used for crosslinking
uuuggucguauugggcgccugg

SEQ ID NO: 452 - RNA, 22 nt, Artificial Sequence
  Nucleic acid sequence used for crosslinking
aggcgcccaauacgaccaaauc

SEQ ID NO: 453 - RNA, 22 nt, Artificial Sequence
  Nucleic acid sequence used for crosslinking
acuuuguuggauuugaaauucc

SEQ ID NO: 454 - RNA, 22 nt, Artificial Sequence
  Nucleic acid sequence used for crosslinking
aauuucaaauccaacaaagucu

SEQ ID NO: 455 - RNA, 21 nt, Artificial Sequence
  Nucleic acid sequence used for crosslinking
gauaagaugaaucucuucucc

SEQ ID NO: 456 - RNA, 21 nt, Artificial Sequence
  Nucleic acid sequence used for crosslinking
agaagagauucaucuuaucuc

SEQ ID NO: 457 - RNA, 22 nt, Artificial Sequence
  Nucleic acid sequence used for crosslinking
uuuggucguauugggcgccugg

SEQ ID NO: 458 - RNA, 22 nt, Artificial Sequence
  Nucleic acid sequence used for crosslinking
aggcgcccaauacgaccaaauc

SEQ ID NO: 459 - RNA, 22 nt, Artificial Sequence
  Nucleic acid sequence used for crosslinking
acuuuguuggauuugaaauucc

SEQ ID NO: 460 - RNA, 22 nt, Artificial Sequence
  Nucleic acid sequence used for crosslinking
aauuucaaauccaacaaagucu

SEQ ID NO: 461 - RNA, 21 nt, Artificial Sequence
  Nucleic acid sequence used for crosslinking
gauaagaugaaucucuucucc

SEQ ID NO: 462 - RNA, 21 nt, Artificial Sequence
  Nucleic acid sequence used for crosslinking
agaagagauucaucuuaucuc

SEQ ID NO: 463 - RNA, 22 nt, Artificial Sequence
  Nucleic acid sequence used for crosslinking
uuuggucguauugggcgccugg

SEQ ID NO: 464 - RNA, 22 nt, Artificial Sequence
  Nucleic acid sequence used for crosslinking
aggcgcccaauacgaccaaauc

SEQ ID NO: 465 - RNA, 22 nt, Artificial Sequence
  Nucleic acid sequence used for crosslinking
acuuuguuggauuugaaauucc

SEQ ID NO: 466 - RNA, 22 nt, Artificial Sequence
  Nucleic acid sequence used for crosslinking
aauuucaaauccaacaaagucu

SEQ ID NO: 467 - RNA, 21 nt, Artificial Sequence
  Nucleic acid sequence used for crosslinking
gauaagaugaaucucuucucc

SEQ ID NO: 468 - RNA, 21 nt, Artificial Sequence
  Nucleic acid sequence used for crosslinking
agaagagauucaucuuaucuc

SEQ ID NO: 469 - RNA, 22 nt, Artificial Sequence
  Nucleic acid sequence used for crosslinking
uuuggucguauugggcgccugg

SEQ ID NO: 470 - RNA, 22 nt, Artificial Sequence
  Nucleic acid sequence used for crosslinking
aggcgcccaauacgaccaaauc

SEQ ID NO: 471 - RNA, 22 nt, Artificial Sequence
  Nucleic acid sequence used for crosslinking
acuuuguuggauuugaaauucc

SEQ ID NO: 472 - RNA, 22 nt, Artificial Sequence
  Nucleic acid sequence used for crosslinking
aauuucaaauccaacaaagucu

SEQ ID NO: 473 - RNA, 21 nt, Artificial Sequence
  Nucleic acid sequence used for crosslinking
gauaagaugaaucucuucucc

SEQ ID NO: 474 - RNA, 21 nt, Artificial Sequence
  Nucleic acid sequence used for crosslinking
agaagagauucaucuuaucuc

SEQ ID NO: 475 - RNA, 22 nt, Artificial Sequence
  Nucleic acid sequence used for crosslinking
uuuggucguauugggcgccugg

SEQ ID NO: 476 - RNA, 22 nt, Artificial Sequence
  Nucleic acid sequence used for crosslinking
aggcgcccaauacgaccaaauc

SEQ ID NO: 477 - RNA, 22 nt, Artificial Sequence
  Nucleic acid sequence used for crosslinking
acuuuguuggauuugaaauucc

SEQ ID NO: 478 - RNA, 22 nt, Artificial Sequence
  Nucleic acid sequence used for crosslinking
aauuucaaauccaacaaagucu

SEQ ID NO: 479 - RNA, 21 nt, Artificial Sequence
  Nucleic acid sequence used for crosslinking
gauaagaugaaucucuucucc

SEQ ID NO: 480 - RNA, 21 nt, Artificial Sequence
  Nucleic acid sequence used for crosslinking
agaagagauucaucuuaucuc

SEQ ID NO: 481 - RNA, 22 nt, Artificial Sequence
  Nucleic acid sequence used for crosslinking
uuuggucguauugggcgccugg

SEQ ID NO: 482 - RNA, 22 nt, Artificial Sequence
  Nucleic acid sequence used for crosslinking
aggcgcccaauacgaccaaauc

SEQ ID NO: 483 - RNA, 22 nt, Artificial Sequence
  Nucleic acid sequence used for crosslinking
acuuuguuggauuugaaauucc

SEQ ID NO: 484 - RNA, 22 nt, Artificial Sequence
  Nucleic acid sequence used for crosslinking
aauuucaaauccaacaaagucu

SEQ ID NO: 485 - RNA, 21 nt, Artificial Sequence
  Nucleic acid sequence used for crosslinking
gauaagaugaaucucuucucc

SEQ ID NO: 486 - RNA, 21 nt, Artificial Sequence
  Nucleic acid sequence used for crosslinking
agaagagauucaucuuaucuc

SEQ ID NO: 487 - RNA, 22 nt, Artificial Sequence
  Nucleic acid sequence used for crosslinking
uuuggucguauugggcgccugg

SEQ ID NO: 488 - RNA, 22 nt, Artificial Sequence
  Nucleic acid sequence used for crosslinking
aggcgcccaauacgaccaaauc

SEQ ID NO: 489 - RNA, 22 nt, Artificial Sequence
  Nucleic acid sequence used for crosslinking
acuuuguuggauuugaaauucc

SEQ ID NO: 490 - RNA, 22 nt, Artificial Sequence
  Nucleic acid sequence used for crosslinking
aauuucaaauccaacaaagucu

SEQ ID NO: 491 - RNA, 21 nt, Artificial Sequence
  Nucleic acid sequence used for crosslinking
gauaagaugaaucucuucucc

SEQ ID NO: 492 - RNA, 21 nt, Artificial Sequence
  Nucleic acid sequence used for crosslinking
agaagagauucaucuuaucuc

SEQ ID NO: 493 - RNA, 22 nt, Artificial Sequence
  Nucleic acid sequence used for crosslinking
uuuggucguauugggcgccugg

SEQ ID NO: 494 - RNA, 22 nt, Artificial Sequence
  Nucleic acid sequence used for crosslinking
aggcgcccaauacgaccaaauc

SEQ ID NO: 495 - RNA, 22 nt, Artificial Sequence
  Nucleic acid sequence used for crosslinking
acuuuguuggauuugaaauucc

SEQ ID NO: 496 - RNA, 22 nt, Artificial Sequence
  Nucleic acid sequence used for crosslinking
aauuucaaauccaacaaagucu

SEQ ID NO: 497 - RNA, 21 nt, Artificial Sequence
  Nucleic acid sequence used for crosslinking
gauaagaugaaucucuucucc

SEQ ID NO: 498 - RNA, 21 nt, Artificial Sequence
  Nucleic acid sequence used for crosslinking
agaagagauucaucuuaucuc

SEQ ID NO: 499 - RNA, 22 nt, Artificial Sequence
  Nucleic acid sequence used for crosslinking
uuuggucguauugggcgccugg

SEQ ID NO: 500 - RNA, 22 nt, Artificial Sequence
  Nucleic acid sequence used for crosslinking
aggcgcccaauacgaccaaauc

SEQ ID NO: 501 - RNA, 22 nt, Artificial Sequence
  Nucleic acid sequence used for crosslinking
acuuuguuggauuugaaauucc

SEQ ID NO: 502 - RNA, 22 nt, Artificial Sequence
  Nucleic acid sequence used for crosslinking
aauuucaaauccaacaaagucu

SEQ ID NO: 503 - RNA, 21 nt, Artificial Sequence
  Nucleic acid sequence used for crosslinking
gauaagaugaaucucuucucc

SEQ ID NO: 504 - RNA, 21 nt, Artificial Sequence
  Nucleic acid sequence used for crosslinking
agaagagauucaucuuaucuc

SEQ ID NO: 505 - RNA, 22 nt, Artificial Sequence
  Nucleic acid sequence used for crosslinking
uuuggucguauugggcgccugg

SEQ ID NO: 506 - RNA, 22 nt, Artificial Sequence
  Nucleic acid sequence used for crosslinking
aggcgcccaauacgaccaaauc

SEQ ID NO: 507 - RNA, 22 nt, Artificial Sequence
  Nucleic acid sequence used for crosslinking
acuuuguuggauuugaaauucc

SEQ ID NO: 508 - RNA, 22 nt, Artificial Sequence
  Nucleic acid sequence used for crosslinking
aauuucaaauccaacaaagucu

SEQ ID NO: 509 - RNA, 21 nt, Artificial Sequence
  Nucleic acid sequence used for crosslinking
gauaagaugaaucucuucucc

SEQ ID NO: 510 - RNA, 21 nt, Artificial Sequence
  Nucleic acid sequence used for crosslinking
agaagagauucaucuuaucuc

SEQ ID NO: 511 - RNA, 22 nt, Artificial Sequence
  Nucleic acid sequence used for crosslinking
uuuggucguauugggcgccugg

SEQ ID NO: 512 - RNA, 22 nt, Artificial Sequence
  Nucleic acid sequence used for crosslinking
aggcgcccaauacgaccaaauc

SEQ ID NO: 513 - RNA, 22 nt, Artificial Sequence
  Nucleic acid sequence used for crosslinking
acuuuguuggauuugaaauucc

SEQ ID NO: 514 - RNA, 22 nt, Artificial Sequence
  Nucleic acid sequence used for crosslinking
aauuucaaauccaacaaagucu

SEQ ID NO: 515 - RNA, 21 nt, Artificial Sequence
  Nucleic acid sequence used for crosslinking
uuggucguauugggcgccugg

SEQ ID NO: 516 - RNA, 21 nt, Artificial Sequence
  Nucleic acid sequence used for crosslinking
aggcgcccaauacgaccaaau

SEQ ID NO: 517 - RNA, 21 nt, Artificial Sequence
  Nucleic acid sequence used for crosslinking
cuuuguuggauuugaaauucc

SEQ ID NO: 518 - RNA, 21 nt, Artificial Sequence
  Nucleic acid sequence used for crosslinking
aauuucaaauccaacaaaguc

SEQ ID NO: 519 - RNA, 21 nt, Artificial Sequence
  Nucleic acid sequence used for crosslinking
uuauggguugggacuacccua

SEQ ID NO: 520 - RNA, 21 nt, Artificial Sequence
  Nucleic acid sequence used for crosslinking
ggguagucccaacccauaagg

SEQ ID NO: 521 - DNA, 20 bp, Artificial Sequence
  primer for amplification of NEK6 gene
ggagttccaacaacctctgc

SEQ ID NO: 522 - DNA, 20 bp, Artificial Sequence
  primer for amplification of NEK6 gene
gagccactgtcttcctgtcc

SEQ ID NO: 523 - DNA, 19 bp, Artificial Sequence
  primer for amplification of GAPDH gene
atggggaaggtgaaggtcg

SEQ ID NO: 524 - DNA, 23 bp, Artificial Sequence
  primer for amplification of GAPDH gene
gggtcattgatggcaacaatatc

SEQ ID NO: 525 - DNA, 21 bp, Artificial Sequence
  primer for amplification of HPRT1 gene
gaaaaggaccccacgaagtgt

SEQ ID NO: 526 - DNA, 23 bp, Artificial Sequence
  primer for amplification of HPRT1 gene
agtcaagggcatatcctacaaca

SEQ ID NO: 527 - DNA, 233 bp, Artificial Sequence
  reporter plasmid Pass 10
ggagaagagattcatcttatctctatatgctgtgtgtactctgctttctagcaccatttgaaatcagtgttagtggcagtgtcttagctggttgtcgcgtaccaaaagtaataatgcgcaaatccgagtccacgtgtggaaataaaccgccagcattcaaggagagaacggctaagaaacttgcccaagaaaacgactcaagtaaggcaagctaccgtggctcgctgaaccac

SEQ ID NO: 528 - DNA, 52 bp, Artificial Sequence
  reporter plasmid GAPDH20-HPRT1
gaccaggcgcccaatacgaccaaatcctggaatttcaaatccaacaaagtct

SEQ ID NO: 529 - DNA, 100 bp, Artificial Sequence
  reporter plasmid SC2013
gttgacaacccttgtcttatgggttgggactaccctaagtgtgatagagcaatggaagggttgtgcctattctggaactgtaatgttgatatgtatcctg

SEQ ID NO: 530 - DNA, 100 bp, Artificial Sequence
  reporter plasmid SAX2011
gttgaaaatccacaccttatgggttgggactatcctaagtgtgaccgtgcaatgaatggtttgtgcctattctggaactgtaacgttgatatgtaccctg

SEQ ID NO: 531 - DNA, 100 bp, Artificial Sequence
  reporter plasmid MERS
gttgataatccgcatcttatgggttgggattaccctaagtgtgatagagctgctgatgggctctgcttattttggaactgtaatgtaccaaaatatccta

SEQ ID NO: 532 - DNA, 100 bp, Artificial Sequence
  reporter plasmid SARS
gtagaaactccacaccttatgggttgggattatccaaaatgtgacagagccactgatggtgtttgtttgttttggaattgtaacgttgatcgttacccag

SEQ ID NO: 533 - DNA, 100 bp, Artificial Sequence
  reporter plasmid HKU3
gtagaaagtcctcacctcatgggttgggactacccaaaatgtgacagagctacagatggcgtgtgtttgttttggaactgtaacgtggatcgttaccctt